European Patent Application EP 4 772 026 A1, published July 8, 2026. Title: セロトニン産生促進用組成物. Applicant: 森永乳業株式会社. Application JP. The sequence listing filed with the application follows.

SEQUENCE LISTING (4 sequences)

SEQ ID NO: 1 - DNA, 23 bp, synthetic construct
  source 1..23: mol_type = other DNA
aacaaagaccattcctccgaaag

SEQ ID NO: 2 - DNA, 23 bp, synthetic construct
  source 1..23: mol_type = other DNA
tgtaacaggctcacatgattctc

SEQ ID NO: 3 - DNA, 20 bp, synthetic construct
  source 1..20: mol_type = other DNA
acattgttgccatcaacgac

SEQ ID NO: 4 - DNA, 20 bp, synthetic construct
  source 1..20: mol_type = other DNA
cttgccgtgggtagcgtcat